European Patent Application EP 4 394 040 A1, published July 3, 2024. Title: A genus of Corynebacterium microorganism for producing L- arginine and a method for producing L-arginine using the same. Applicant: CJ CheilJedang Corporation. The sequence listing filed with the application follows.

SEQUENCE LISTING (16 sequences)

SEQ ID NO: 1 - protein, 203 aa, Corynebacterium
  REGION 1..203: note = NCgl1469 amino acid sequence
MSPTVLPATQADFPKIVDVLVEAFANDPAFLRWIPQPDPGSAKLRALFELQIEKQYAVAGNIDVARDSEGEIVGVALWDRPDGNHSAKDQAAILPRLVSIFGIKAAQVAWTDLSSARFHPKFPHWYLYTVATSSSARGTGVGSALLNHGIARAGDEAIYLEATSTRAAQLYNRLGFVPLGYIPSDDDGTPELAMWKPPAMPTV

SEQ ID NO: 2 - DNA, 612 bp, Corynebacterium
  misc_feature 1..612: note = NCgl1469 nucleotide sequence
  source 1..612: mol_type = genomic DNA
atgagtcccaccgttttgcctgctacacaagctgacttccctaagatcgtcgatgttctggttgaagcattcgccaacgatccagcatttttacgatggatcccgcagccggaccccggttcagcaaagcttcgagcacttttcgaactgcagattgagaagcagtatgcagtggcgggaaatattgatgtcgcgcgtgattctgagggagaaatcgtcggcgtcgcgttatgggatcggccagatggtaatcacagtgccaaagatcaagcagcgatactcccccggctcgtctccattttcgggatcaaggctgcgcaggtggcgtggacggatttgagttcggctcgtttccaccccaaattcccccattggtacctctacaccgtggcaacatctagttctgcccgtggaacgggtgttggcagtgcgcttcttaatcacggaatcgctcgcgcgggtgatgaagctatctatttggaggcgacgtcgactcgtgcggctcaactatataaccgtctgggatttgtgcccttgggttatatcccctcagatgatgatggcactcctgaactggcgatgtggaaaccgccagcgatgccaactgtttaa

SEQ ID NO: 3 - DNA, 25 bp, synthetic construct
  misc_feature 1..25: note = primer 1
  source 1..25: mol_type = other DNA
acctacaacaaagctctcatcaacc

SEQ ID NO: 4 - DNA, 24 bp, synthetic construct
  misc_feature 1..24: note = primer 2
  source 1..24: mol_type = other DNA
ctaccctgtggaacacctacatct

SEQ ID NO: 5 - DNA, 34 bp, synthetic construct
  misc_feature 1..34: note = primer 3
  source 1..34: mol_type = other DNA
tcgagctcggtaccctcagtgctccaactgcttg

SEQ ID NO: 6 - DNA, 34 bp, synthetic construct
  misc_feature 1..34: note = primer 4
  source 1..34: mol_type = other DNA
cttcagggggataccagaatagcgaaatgaaaag

SEQ ID NO: 7 - DNA, 34 bp, synthetic construct
  misc_feature 1..34: note = primer 5
  source 1..34: mol_type = other DNA
ctggtatccccctgaaggcgatttaaggggtcga

SEQ ID NO: 8 - DNA, 34 bp, synthetic construct
  misc_feature 1..34: note = primer 6
  source 1..34: mol_type = other DNA
ctctagaggatccccgcaggggagtttgaaaaac

SEQ ID NO: 9 - DNA, 34 bp, synthetic construct
  misc_feature 1..34: note = primer 7
  source 1..34: mol_type = other DNA
tcgagctcggtacccagcaggccttaagggtaag

SEQ ID NO: 10 - DNA, 34 bp, synthetic construct
  misc_feature 1..34: note = primer 8
  source 1..34: mol_type = other DNA
aggggcgctgtcttacctcggctggtgggccagc

SEQ ID NO: 11 - DNA, 36 bp, synthetic construct
  misc_feature 1..36: note = primer 9
  source 1..36: mol_type = other DNA
ggtaagacagcgcccctagttcaaggcttgttaatc

SEQ ID NO: 12 - DNA, 35 bp, synthetic construct
  misc_feature 1..35: note = primer 10
  source 1..35: mol_type = other DNA
ctctagaggatccccaccgttgaactgcttgccag

SEQ ID NO: 13 - protein, 171 aa, Corynebacterium
  REGION 1..171: note = argR amino acid sequence
MSLGSTPSTPENLNPVTRTARQALILQILDKQKVTSQVQLSELLLDEGIDITQATLSRDLDELGARKVRPDGGRAYYAVGPVDSIAREDLRGPSEKLRRMLDELLVSTDHSGNIAMLRTPPGAAQYLASFIDRVGLKEVVGTIAGDDTVFVLARDPLTGKELGELLSGRTT

SEQ ID NO: 14 - DNA, 516 bp, Corynebacterium
  misc_feature 1..516: note = argR nucleotide sequence
  source 1..516: mol_type = genomic DNA
atgtcccttggctcaaccccgtcaacaccggaaaacttaaatcccgtgactcgcactgcacgccaagctctcattttgcagattttggacaaacaaaaagtcaccagccaggtacaactgtctgaattgctgctggatgaaggcatcgatatcacccaggccaccttgtcccgagatctcgatgaactcggtgcacgcaaggttcgccccgatgggggacgcgcctactacgcggtcggcccagtagatagcatcgcccgcgaagatctccggggtccgtcggagaagctgcgccgcatgcttgatgaactgctggtttctacagatcattccggcaacatcgcgatgctgcgcaccccgccgggagctgcccagtacctggcaagtttcatcgatagggtggggctgaaagaagtcgttggcaccatcgctggcgatgacaccgttttcgttctcgcccgtgatccgctcacaggtaaagaactaggtgaattactcagcgggcgcaccacttaa

SEQ ID NO: 15 - protein, 319 aa, Corynebacterium
  REGION 1..319: note = argF amino acid sequence
MTSQPQVRHFLADDDLTPAEQAEVLTLAAKLKAAPFSERPLEGPKSVAVLFDKTSTRTRFSFDAGIAHLGGHAIVVDSGSSQMGKGETLQDTAAVLSRYVEAIVWRTYAHSNFHAMAETSTVPLVNSLSDDLHPCQILADLQTIVENLSPEEGPAGLKGKKAVYLGDGDNNMANSYMIGFATAGMDISIIAPEGFQPRAEFVERAEKRGQETGAKVVVTDSLDEVAGADVVITDTWVSMGMENDGIDRTTPFVPYQVNDEVMAKANDGAIFLHCLPAYRGKEVAASVIDGPASKVFDEAENRLHAQKALLVWLLAHQPR

SEQ ID NO: 16 - DNA, 960 bp, Corynebacterium
  misc_feature 1..960: note = argF nucleotide sequence
  source 1..960: mol_type = genomic DNA
atgacttcacaaccacaggttcgccatttcctggctgatgatgatctcacccctgcagagcaggcagaggttttgaccctagccgcaaagctcaaggcagcgccgttttcggagcgtccactcgagggaccaaagtccgttgcagttctttttgataagacttcaactcgtactcgcttctccttcgacgcgggcatcgctcatttgggtggacatgccatcgtcgtggattccggcagctcacagatgggtaagggcgagaccctgcaggacaccgcagctgtattgtcccgctacgtggaagcaattgtgtggcgcacctacgcacacagcaatttccacgccatggcggagacgtccactgtgccactggtgaactccttgtccgatgatctgcacccatgccagattctggctgatctgcagaccatcgtggaaaacctcagccctgaagaaggcccagcaggccttaagggtaagaaggctgtgtacctgggcgatggcgacaacaacatggccaactcctacatgattggctttgccaccgcgggcatggatatctccatcatcgctcctgaagggttccagcctcgtgcggaattcgtggagcgcgcggaaaagcgtggccaggaaaccggcgcgaaggttgttgtcaccgacagcctcgacgaggttgccggcgccgatgttgtcatcaccgatacctgggtatccatgggtatggaaaacgacggcatcgatcgcaccacacctttcgttccctaccaggtcaacgatgaggtcatggcgaaagctaacgacggcgccatcttcctgcactgccttcctgcctaccgcggcaaagaagtggcagcctccgtgattgatggaccagcgtccaaagttttcgatgaagcagaaaaccgcctccacgctcagaaagcactgctggtgtggctgctggcccaccagccgaggtaa